European Patent Application EP 4 796 632 A1, published August 26, 2026. Title: Improved synthesis of a puromycin linker. Applicant: Deutsches Krebsforschungszentrum Stiftung des öffentlichen Rechts. Application EP. The sequence listing filed with the application follows.

SEQUENCE LISTING (19 sequences)

SEQ ID NO: 1 - DNA, 20 bp, synthetic construct
  source 1..20: mol_type = other DNA
aatttccacgccgccccccg

SEQ ID NO: 2 - DNA, 24 bp, synthetic construct
  source 1..24: mol_type = other DNA
  modified_base 21: mod_base = OTHER; note = linker L3 - functional group FGb
aatttccacgccgccccccgtcct

SEQ ID NO: 3 - DNA, 20 bp, synthetic construct
  source 1..20: mol_type = other DNA
  modified_base 10: mod_base = OTHER; note = Cyanovinylcarbazole nucleotide
aatttccangccgccccccg

SEQ ID NO: 4 - DNA, 23 bp, synthetic construct
  source 1..23: mol_type = other DNA
  misc_feature 3: note = optional ribonucleotide
  modified_base 12: mod_base = OTHER; note = Cyanovinylcarbazole nucleotide
aagaatttccangccgccccccg

SEQ ID NO: 5 - DNA, 24 bp, synthetic construct
  source 1..24: mol_type = other DNA
  modified_base 9: mod_base = OTHER; note = Cyanovinylcarbazole nucleotide
  modified_base 21: mod_base = OTHER; note = linker L3 - functional group FGb
aatttccangccgccccccgtcct

SEQ ID NO: 6 - DNA, 27 bp, synthetic construct
  source 1..27: mol_type = other DNA
  misc_feature 3: note = optional ribonucleotide
  modified_base 12: mod_base = OTHER; note = Cyanovinylcarbazole nucleotide
  modified_base 24: mod_base = OTHER; note = linker L3 - functional group FGb
aagaatttccangccgccccccgtcct

SEQ ID NO: 7 - DNA, 27 bp, synthetic construct
  source 1..27: mol_type = other DNA
  misc_feature 3: note = optional ribonucleotide
  modified_base 12: mod_base = OTHER; note = Cyanovinylcarbazole nucleotide
  modified_base 24: mod_base = OTHER; note = linker L3 - functional group FGb
  modified_base 6: mod_base = OTHER; note = fluorescein
aagaatttccangccgccccccgtcct

SEQ ID NO: 8 - DNA, 28 bp, synthetic construct
  source 1..28: mol_type = other DNA
  misc_feature 4: note = optional ribonucleotide
  modified_base 1: mod_base = OTHER; note = gamma-[N-(Biotin-6-amino-hexanoyl)]-5-propargylamino-2',3'-dideoxyuridine
  modified_base 12: mod_base = OTHER; note = Cyanovinylcarbazole nucleotide
  modified_base 25: mod_base = OTHER; note = linker L3 - functional group FGb
taagaatttccangccgccccccgtcct

SEQ ID NO: 9 - protein, 25 aa, synthetic construct
MGGACYSVVCHVWMICGSGHHHHHH

SEQ ID NO: 10 - protein, 30 aa, synthetic construct
MGGACYSVVCHVWMICGSGHHHHHHGKLGG

SEQ ID NO: 11 - protein, 26 aa, synthetic construct
MGGACYSVVCHVWMICGSGHHHHHHG

SEQ ID NO: 12 - DNA, 28 bp, synthetic construct
  source 1..28: mol_type = other DNA
  modified_base 1: mod_base = OTHER; note = dT-Biotin
  misc_feature 3: note = optional ribonucleotide
  modified_base 24: mod_base = OTHER; note = linkerL3 - functional group Fgb
  modified_base 6: mod_base = OTHER; note = fluorescin
taagaatttccangccgccccccgtcct

SEQ ID NO: 13 - DNA, 28 bp, synthetic construct
  source 1..28: mol_type = other DNA
  misc_feature 3: note = otional ribonucleotide
  modified_base 1: mod_base = OTHER; note = dT-Biotin
  modified_base 12: mod_base = OTHER; note = Cyanovinylcarbazole nucleotide
  modified_base 24: mod_base = OTHER; note = linker L3 - functional group FGb
taagaatttccangccgccccccgtcct

SEQ ID NO: 14 - protein, 26 aa, synthetic construct
  MOD_RES 26: note = -puromycin-cytosine-cytosine
MGGACYSVVCHVMWICGSGHHHHHHG

SEQ ID NO: 15 - DNA, 27 bp, synthetic construct
  source 1..27: mol_type = other DNA
  modified_base 1: mod_base = OTHER; note = Biotin-TEG-
  modified_base 12: mod_base = OTHER; note = CNVK
  modified_base 3: mod_base = OTHER; note = optional ribonucleotide
  modified_base 6: mod_base = OTHER; note = fluorescein
  modified_base 24: mod_base = OTHER; note = DBCO-C6-
aagaatttccangccgccccccgtcct

SEQ ID NO: 16 - DNA, 20 bp, synthetic construct
  source 1..20: mol_type = other DNA
ttactcgctccatgggcggc

SEQ ID NO: 17 - DNA, 37 bp, synthetic construct
  source 1..37: mol_type = other DNA
ataatcttaagctttccatgatgatgatgatgatggc

SEQ ID NO: 18 - DNA, 76 bp, synthetic construct
  source 1..76: mol_type = other DNA
atgggcggcgcgtgttactctgttgtttgtcatgtttggatgatctgtggcagcggccatcatcatcatcatcatg

SEQ ID NO: 19 - protein, 25 aa, synthetic construct
MGGACYSVVCHVWMICGSGHHHHHH